European Patent Application EP 4 803 540 A1, published September 9, 2026. Title: Novel functions of CSF3 inhibitors and a use thereof. Applicant: FNCT Biotech, Inc. The sequence listing filed with the application follows.

SEQUENCE LISTING (163 sequences)

SEQ ID NO: 1 - protein, 8 aa, synthetic construct
  source 1..8: note = CDRH1 of anti-CSF3 antibody
GYTFTNYG

SEQ ID NO: 2 - protein, 8 aa, synthetic construct
  source 1..8: note = CDRH2 of anti-CSF3 antibody
INPNSGGT

SEQ ID NO: 3 - protein, 12 aa, synthetic construct
  source 1..12: note = CDRH3 of anti-CSF3 antibody
SRGSGGRDAFDV

SEQ ID NO: 4 - protein, 12 aa, synthetic construct
  source 1..12: note = CDRH3 of anti-CSF3 antibody
SRGSGGHLAFDV

SEQ ID NO: 5 - protein, 12 aa, synthetic construct
  source 1..12: note = CDRH3 of anti-CSF3 antibody
SRGSGGMSGFDV

SEQ ID NO: 6 - protein, 12 aa, synthetic construct
  source 1..12: note = CDRH3 of anti-CSF3 antibody
SRGSGGRNGFDV

SEQ ID NO: 7 - protein, 12 aa, synthetic construct
  source 1..12: note = CDRH3 of anti-CSF3 antibody
SRGSGGTTGFDV

SEQ ID NO: 8 - protein, 12 aa, synthetic construct
  source 1..12: note = CDRH3 of anti-CSF3 antibody
SRGSGGMHPFDV

SEQ ID NO: 9 - protein, 12 aa, synthetic construct
  source 1..12: note = CDRH3 of anti-CSF3 antibody
SRGSGGTSPFDV

SEQ ID NO: 10 - protein, 12 aa, synthetic construct
  source 1..12: note = CDRH3 of anti-CSF3 antibody
SRGSGGIKPFDV

SEQ ID NO: 11 - protein, 12 aa, synthetic construct
  source 1..12: note = CDRH3 of anti-CSF3 antibody
SRGSGGAVPFDV

SEQ ID NO: 12 - protein, 12 aa, synthetic construct
  source 1..12: note = CDRH3 of anti-CSF3 antibody
SRGSGGIAPFDV

SEQ ID NO: 13 - protein, 12 aa, synthetic construct
  source 1..12: note = CDRH3 of anti-CSF3 antibody
SRGSGGLLPFDV

SEQ ID NO: 14 - protein, 12 aa, synthetic construct
  source 1..12: note = CDRH3 of anti-CSF3 antibody
SRGSGGMVPFDV

SEQ ID NO: 15 - protein, 12 aa, synthetic construct
  source 1..12: note = CDRH3 of anti-CSF3 antibody
SRGSGGRSGFDV

SEQ ID NO: 16 - protein, 12 aa, synthetic construct
  source 1..12: note = CDRH3 of anti-CSF3 antibody
SRGSGGFQAFDV

SEQ ID NO: 17 - protein, 12 aa, synthetic construct
  source 1..12: note = CDRH3 of anti-CSF3 antibody
SRGSGGLVPFDV

SEQ ID NO: 18 - protein, 12 aa, synthetic construct
  source 1..12: note = CDRH3 of anti-CSF3 antibody
SRGSGGIRPFDV

SEQ ID NO: 19 - protein, 12 aa, synthetic construct
  source 1..12: note = CDRH3 of anti-CSF3 antibody
SRGSGGFFPFDV

SEQ ID NO: 20 - protein, 12 aa, synthetic construct
  source 1..12: note = CDRH3 of anti-CSF3 antibody
SRGSGGYSGFDV

SEQ ID NO: 21 - protein, 6 aa, synthetic construct
  source 1..6: note = CDRL1 of anti-CSF3 antibody
QTISTY

SEQ ID NO: 22 - protein, 6 aa, synthetic construct
  source 1..6: note = CDRL1 of anti-CSF3 antibody
QTTGQY

SEQ ID NO: 23 - protein, 6 aa, synthetic construct
  source 1..6: note = CDRL1 of anti-CSF3 antibody
QTISNR

SEQ ID NO: 24 - protein, 6 aa, synthetic construct
  source 1..6: note = CDRL1 of anti-CSF3 antibody
KSISTY

SEQ ID NO: 25 - skipped

SEQ ID NO: 26 - protein, 9 aa, synthetic construct
  source 1..9: note = CDRL3 of anti-CSF3 antibody
QQGYSSPRT

SEQ ID NO: 27 - protein, 25 aa, synthetic construct
  source 1..25: note = FRH1 of anti-CSF3 antibody
QMQLVQSGAEARKPGSSVKVSCKAS

SEQ ID NO: 28 - protein, 25 aa, synthetic construct
  source 1..25: note = FRH1 of anti-CSF3 antibody
EMQLVQSGAEARKPGSSVKVSCKAS

SEQ ID NO: 29 - protein, 17 aa, synthetic construct
  source 1..17: note = FRH2 of anti-CSF3 antibody
ISWLRQTPGQGLEWMGW

SEQ ID NO: 30 - protein, 38 aa, synthetic construct
  source 1..38: note = FRH3 of anti-CSF3 antibody
IYAQKFQGRVTMTRDTSITTAYMELSTLRSEDTAVYYC

SEQ ID NO: 31 - protein, 38 aa, synthetic construct
  source 1..38: note = FRH3 of anti-CSF3 antibody
IYAQKFQGRVTMTRDTPITTAYMELSTLRSEDTAVYYC

SEQ ID NO: 32 - protein, 11 aa, synthetic construct
  source 1..11: note = FRH4 of anti-CSF3 antibody
WGQGTMVTVSS

SEQ ID NO: 33 - protein, 26 aa, synthetic construct
  source 1..26: note = FRL1 of anti-CSF3 antibody
DIQMTQSPFSLSASVGDRVTITCRAS

SEQ ID NO: 34 - protein, 17 aa, synthetic construct
  source 1..17: note = FRL2 of anti-CSF3 antibody
LNWYQHKPGKAPKLFIY

SEQ ID NO: 35 - protein, 36 aa, synthetic construct
  source 1..36: note = FRL3 of anti-CSF3 antibody
SLQSGVPSRFSGSGSGTDFALTISSLQPEDFATYYC

SEQ ID NO: 36 - protein, 10 aa, synthetic construct
  source 1..10: note = FRL4 of anti-CSF3 antibody
FGQGTKVEIK

SEQ ID NO: 37 - protein, 10 aa, synthetic construct
  source 1..10: note = FRL4 of anti-CSF3 antibody
FGQGTKVEIT

SEQ ID NO: 38 - protein, 119 aa, synthetic construct
  source 1..119: note = VH of anti-CSF3 antibody
QMQLVQSGAEARKPGSSVKVSCKASGYTFTNYGISWLRQTPGQGLEWMGWINPNSGGTIYAQKFQGRVTMTRDTSITTAYMELSTLRSEDTAVYYCSRGSGGRDAFDVWGQGTMVTVSS

SEQ ID NO: 39 - protein, 119 aa, synthetic construct
  source 1..119: note = VH of anti-CSF3 antibody
QMQLVQSGAEARKPGSSVKVSCKASGYTFTNYGISWLRQTPGQGLEWMGWINPNSGGTIYAQKFQGRVTMTRDTSITTAYMELSTLRSEDTAVYYCSRGSGGHLAFDVWGQGTMVTVSS

SEQ ID NO: 40 - protein, 119 aa, synthetic construct
  source 1..119: note = VH of anti-CSF3 antibody
QMQLVQSGAEARKPGSSVKVSCKASGYTFTNYGISWLRQTPGQGLEWMGWINPNSGGTIYAQKFQGRVTMTRDTSITTAYMELSTLRSEDTAVYYCSRGSGGMSGFDVWGQGTMVTVSS

SEQ ID NO: 41 - protein, 119 aa, synthetic construct
  source 1..119: note = VH of anti-CSF3 antibody
QMQLVQSGAEARKPGSSVKVSCKASGYTFTNYGISWLRQTPGQGLEWMGWINPNSGGTIYAQKFQGRVTMTRDTSITTAYMELSTLRSEDTAVYYCSRGSGGRNGFDVWGQGTMVTVSS

SEQ ID NO: 42 - protein, 119 aa, synthetic construct
  source 1..119: note = VH of anti-CSF3 antibody
QMQLVQSGAEARKPGSSVKVSCKASGYTFTNYGISWLRQTPGQGLEWMGWINPNSGGTIYAQKFQGRVTMTRDTSITTAYMELSTLRSEDTAVYYCSRGSGGTTGFDVWGQGTMVTVSS

SEQ ID NO: 43 - protein, 119 aa, synthetic construct
  source 1..119: note = VH of anti-CSF3 antibody
QMQLVQSGAEARKPGSSVKVSCKASGYTFTNYGISWLRQTPGQGLEWMGWINPNSGGTIYAQKFQGRVTMTRDTSITTAYMELSTLRSEDTAVYYCSRGSGGMHPFDVWGQGTMVTVSS

SEQ ID NO: 44 - protein, 119 aa, synthetic construct
  source 1..119: note = VH of anti-CSF3 antibody
QMQLVQSGAEARKPGSSVKVSCKASGYTFTNYGISWLRQTPGQGLEWMGWINPNSGGTIYAQKFQGRVTMTRDTSITTAYMELSTLRSEDTAVYYCSRGSGGTSPFDVWGQGTMVTVSS

SEQ ID NO: 45 - protein, 119 aa, synthetic construct
  source 1..119: note = VH of anti-CSF3 antibody
QMQLVQSGAEARKPGSSVKVSCKASGYTFTNYGISWLRQTPGQGLEWMGWINPNSGGTIYAQKFQGRVTMTRDTSITTAYMELSTLRSEDTAVYYCSRGSGGIKPFDVWGQGTMVTVSS

SEQ ID NO: 46 - protein, 119 aa, synthetic construct
  source 1..119: note = VH of anti-CSF3 antibody
EMQLVQSGAEARKPGSSVKVSCKASGYTFTNYGISWLRQTPGQGLEWMGWINPNSGGTIYAQKFQGRVTMTRDTPITTAYMELSTLRSEDTAVYYCSRGSGGAVPFDVWGQGTMVTVSS

SEQ ID NO: 47 - protein, 119 aa, synthetic construct
  source 1..119: note = VH of anti-CSF3 antibody
QMQLVQSGAEARKPGSSVKVSCKASGYTFTNYGISWLRQTPGQGLEWMGWINPNSGGTIYAQKFQGRVTMTRDTSITTAYMELSTLRSEDTAVYYCSRGSGGIAPFDVWGQGTMVTVSS

SEQ ID NO: 48 - protein, 119 aa, synthetic construct
  source 1..119: note = VH of anti-CSF3 antibody
QMQLVQSGAEARKPGSSVKVSCKASGYTFTNYGISWLRQTPGQGLEWMGWINPNSGGTIYAQKFQGRVTMTRDTSITTAYMELSTLRSEDTAVYYCSRGSGGLLPFDVWGQGTMVTVSS

SEQ ID NO: 49 - protein, 119 aa, synthetic construct
  source 1..119: note = VH of anti-CSF3 antibody
QMQLVQSGAEARKPGSSVKVSCKASGYTFTNYGISWLRQTPGQGLEWMGWINPNSGGTIYAQKFQGRVTMTRDTSITTAYMELSTLRSEDTAVYYCSRGSGGMVPFDVWGQGTMVTVSS

SEQ ID NO: 50 - protein, 119 aa, synthetic construct
  source 1..119: note = VH of anti-CSF3 antibody
QMQLVQSGAEARKPGSSVKVSCKASGYTFTNYGISWLRQTPGQGLEWMGWINPNSGGTIYAQKFQGRVTMTRDTSITTAYMELSTLRSEDTAVYYCSRGSGGRSGFDVWGQGTMVTVSS

SEQ ID NO: 51 - protein, 119 aa, synthetic construct
  source 1..119: note = VH of anti-CSF3 antibody
QMQLVQSGAEARKPGSSVKVSCKASGYTFTNYGISWLRQTPGQGLEWMGWINPNSGGTIYAQKFQGRVTMTRDTSITTAYMELSTLRSEDTAVYYCSRGSGGFQAFDVWGQGTMVTVSS

SEQ ID NO: 52 - protein, 119 aa, synthetic construct
  source 1..119: note = VH of anti-CSF3 antibody
QMQLVQSGAEARKPGSSVKVSCKASGYTFTNYGISWLRQTPGQGLEWMGWINPNSGGTIYAQKFQGRVTMTRDTSITTAYMELSTLRSEDTAVYYCSRGSGGLVPFDVWGQGTMVTVSS

SEQ ID NO: 53 - protein, 119 aa, synthetic construct
  source 1..119: note = VH of anti-CSF3 antibody
QMQLVQSGAEARKPGSSVKVSCKASGYTFTNYGISWLRQTPGQGLEWMGWINPNSGGTIYAQKFQGRVTMTRDTSITTAYMELSTLRSEDTAVYYCSRGSGGIRPFDVWGQGTMVTVSS

SEQ ID NO: 54 - protein, 119 aa, synthetic construct
  source 1..119: note = VH of anti-CSF3 antibody
QMQLVQSGAEARKPGSSVKVSCKASGYTFTNYGISWLRQTPGQGLEWMGWINPNSGGTIYAQKFQGRVTMTRDTSITTAYMELSTLRSEDTAVYYCSRGSGGFFPFDVWGQGTMVTVSS

SEQ ID NO: 55 - protein, 119 aa, synthetic construct
  source 1..119: note = VH of anti-CSF3 antibody
QMQLVQSGAEARKPGSSVKVSCKASGYTFTNYGISWLRQTPGQGLEWMGWINPNSGGTIYAQKFQGRVTMTRDTSITTAYMELSTLRSEDTAVYYCSRGSGGYSGFDVWGQGTMVTVSS

SEQ ID NO: 56 - protein, 107 aa, synthetic construct
  source 1..107: note = VL of anti-CSF3 antibody
DIQMTQSPFSLSASVGDRVTITCRASQTISTYLNWYQHKPGKAPKLFIYYASSLQSGVPSRFSGSGSGTDFALTISSLQPEDFATYYCQQGYSSPRTFGQGTKVEIK

SEQ ID NO: 57 - protein, 107 aa, synthetic construct
  source 1..107: note = VL of anti-CSF3 antibody
DIQMTQSPFSLSASVGDRVTITCRASQTISTYLNWYQHKPGKAPKLFIYYASSLQSGVPSRFSGSGSGTDFALTISSLQPEDFATYYCQQGYSSPRTFGQGTKVEIT

SEQ ID NO: 58 - protein, 107 aa, synthetic construct
  source 1..107: note = VL of anti-CSF3 antibody
DIQMTQSPFSLSASVGDRVTITCRASQTTGQYLNWYQHKPGKAPKLFIYYASSLQSGVPSRFSGSGSGTDFALTISSLQPEDFATYYCQQGYSSPRTFGQGTKVEIK

SEQ ID NO: 59 - protein, 107 aa, synthetic construct
  source 1..107: note = VL of anti-CSF3 antibody
DIQMTQSPFSLSASVGDRVTITCRASQTISNRLNWYQHKPGKAPKLFIYYASSLQSGVPSRFSGSGSGTDFALTISSLQPEDFATYYCQQGYSSPRTFGQGTKVEIK

SEQ ID NO: 60 - protein, 107 aa, synthetic construct
  source 1..107: note = VL of anti-CSF3 antibody
DIQMTQSPFSLSASVGDRVTITCRASKSISTYLNWYQHKPGKAPKLFIYYASSLQSGVPSRFSGSGSGTDFALTISSLQPEDFATYYCQQGYSSPRTFGQGTKVEIK

SEQ ID NO: 61 - protein, 330 aa, synthetic construct
  source 1..330: note = CH of anti-CSF3 antibody
ASTKGPSVFPLAPSSKSTSGGTAALGCLVKDYFPEPVTVSWNSGALTSGVHTFPAVLQSSGLYSLSSVVTVPSSSLGTQTYICNVNHKPSNTKVDKKVEPKSCDKTHTCPPCPAPELLGGPSVFLFPPKPKDTLMISRTPEVTCVVVDVSHEDPEVKFNWYVDGVEVHNAKTKPREEQYNSTYRVVSVLTVLHQDWLNGKEYKCKVSNKALPAPIEKTISKAKGQPREPQVYTLPPSREEMTKNQVSLTCLVKGFYPSDIAVEWESNGQPENNYKTTPPVLDSDGSFFLYSKLTVDKSRWQQGNVFSCSVMHEALHNHYTQKSLSLSPGK

SEQ ID NO: 62 - protein, 107 aa, synthetic construct [sequence omitted]

SEQ ID NO: 63 - protein, 449 aa, synthetic construct
  source 1..449: note = heavy chain of anti-CSF3 antibody
QMQLVQSGAEARKPGSSVKVSCKASGYTFTNYGISWLRQTPGQGLEWMGWINPNSGGTIYAQKFQGRVTMTRDTSITTAYMELSTLRSEDTAVYYCSRGSGGRDAFDVWGQGTMVTVSSASTKGPSVFPLAPSSKSTSGGTAALGCLVKDYFPEPVTVSWNSGALTSGVHTFPAVLQSSGLYSLSSVVTVPSSSLGTQTYICNVNHKPSNTKVDKKVEPKSCDKTHTCPPCPAPELLGGPSVFLFPPKPKDTLMISRTPEVTCVVVDVSHEDPEVKFNWYVDGVEVHNAKTKPREEQYNSTYRVVSVLTVLHQDWLNGKEYKCKVSNKALPAPIEKTISKAKGQPREPQVYTLPPSREEMTKNQVSLTCLVKGFYPSDIAVEWESNGQPENNYKTTPPVLDSDGSFFLYSKLTVDKSRWQQGNVFSCSVMHEALHNHYTQKSLSLSPGK

SEQ ID NO: 64 - protein, 449 aa, synthetic construct
  source 1..449: note = heavy chain of anti-CSF3 antibody
QMQLVQSGAEARKPGSSVKVSCKASGYTFTNYGISWLRQTPGQGLEWMGWINPNSGGTIYAQKFQGRVTMTRDTSITTAYMELSTLRSEDTAVYYCSRGSGGHLAFDVWGQGTMVTVSSASTKGPSVFPLAPSSKSTSGGTAALGCLVKDYFPEPVTVSWNSGALTSGVHTFPAVLQSSGLYSLSSVVTVPSSSLGTQTYICNVNHKPSNTKVDKKVEPKSCDKTHTCPPCPAPELLGGPSVFLFPPKPKDTLMISRTPEVTCVVVDVSHEDPEVKFNWYVDGVEVHNAKTKPREEQYNSTYRVVSVLTVLHQDWLNGKEYKCKVSNKALPAPIEKTISKAKGQPREPQVYTLPPSREEMTKNQVSLTCLVKGFYPSDIAVEWESNGQPENNYKTTPPVLDSDGSFFLYSKLTVDKSRWQQGNVFSCSVMHEALHNHYTQKSLSLSPGK

SEQ ID NO: 65 - protein, 449 aa, synthetic construct
  source 1..449: note = heavy chain of anti-CSF3 antibody
QMQLVQSGAEARKPGSSVKVSCKASGYTFTNYGISWLRQTPGQGLEWMGWINPNSGGTIYAQKFQGRVTMTRDTSITTAYMELSTLRSEDTAVYYCSRGSGGMSGFDVWGQGTMVTVSSASTKGPSVFPLAPSSKSTSGGTAALGCLVKDYFPEPVTVSWNSGALTSGVHTFPAVLQSSGLYSLSSVVTVPSSSLGTQTYICNVNHKPSNTKVDKKVEPKSCDKTHTCPPCPAPELLGGPSVFLFPPKPKDTLMISRTPEVTCVVVDVSHEDPEVKFNWYVDGVEVHNAKTKPREEQYNSTYRVVSVLTVLHQDWLNGKEYKCKVSNKALPAPIEKTISKAKGQPREPQVYTLPPSREEMTKNQVSLTCLVKGFYPSDIAVEWESNGQPENNYKTTPPVLDSDGSFFLYSKLTVDKSRWQQGNVFSCSVMHEALHNHYTQKSLSLSPGK

SEQ ID NO: 66 - protein, 449 aa, synthetic construct
  source 1..449: note = heavy chain of anti-CSF3 antibody
QMQLVQSGAEARKPGSSVKVSCKASGYTFTNYGISWLRQTPGQGLEWMGWINPNSGGTIYAQKFQGRVTMTRDTSITTAYMELSTLRSEDTAVYYCSRGSGGRNGFDVWGQGTMVTVSSASTKGPSVFPLAPSSKSTSGGTAALGCLVKDYFPEPVTVSWNSGALTSGVHTFPAVLQSSGLYSLSSVVTVPSSSLGTQTYICNVNHKPSNTKVDKKVEPKSCDKTHTCPPCPAPELLGGPSVFLFPPKPKDTLMISRTPEVTCVVVDVSHEDPEVKFNWYVDGVEVHNAKTKPREEQYNSTYRVVSVLTVLHQDWLNGKEYKCKVSNKALPAPIEKTISKAKGQPREPQVYTLPPSREEMTKNQVSLTCLVKGFYPSDIAVEWESNGQPENNYKTTPPVLDSDGSFFLYSKLTVDKSRWQQGNVFSCSVMHEALHNHYTQKSLSLSPGK

SEQ ID NO: 67 - protein, 449 aa, synthetic construct
  source 1..449: note = heavy chain of anti-CSF3 antibody
QMQLVQSGAEARKPGSSVKVSCKASGYTFTNYGISWLRQTPGQGLEWMGWINPNSGGTIYAQKFQGRVTMTRDTSITTAYMELSTLRSEDTAVYYCSRGSGGTTGFDVWGQGTMVTVSSASTKGPSVFPLAPSSKSTSGGTAALGCLVKDYFPEPVTVSWNSGALTSGVHTFPAVLQSSGLYSLSSVVTVPSSSLGTQTYICNVNHKPSNTKVDKKVEPKSCDKTHTCPPCPAPELLGGPSVFLFPPKPKDTLMISRTPEVTCVVVDVSHEDPEVKFNWYVDGVEVHNAKTKPREEQYNSTYRVVSVLTVLHQDWLNGKEYKCKVSNKALPAPIEKTISKAKGQPREPQVYTLPPSREEMTKNQVSLTCLVKGFYPSDIAVEWESNGQPENNYKTTPPVLDSDGSFFLYSKLTVDKSRWQQGNVFSCSVMHEALHNHYTQKSLSLSPGK

SEQ ID NO: 68 - protein, 449 aa, synthetic construct
  source 1..449: note = heavy chain of anti-CSF3 antibody
QMQLVQSGAEARKPGSSVKVSCKASGYTFTNYGISWLRQTPGQGLEWMGWINPNSGGTIYAQKFQGRVTMTRDTSITTAYMELSTLRSEDTAVYYCSRGSGGMHPFDVWGQGTMVTVSSASTKGPSVFPLAPSSKSTSGGTAALGCLVKDYFPEPVTVSWNSGALTSGVHTFPAVLQSSGLYSLSSVVTVPSSSLGTQTYICNVNHKPSNTKVDKKVEPKSCDKTHTCPPCPAPELLGGPSVFLFPPKPKDTLMISRTPEVTCVVVDVSHEDPEVKFNWYVDGVEVHNAKTKPREEQYNSTYRVVSVLTVLHQDWLNGKEYKCKVSNKALPAPIEKTISKAKGQPREPQVYTLPPSREEMTKNQVSLTCLVKGFYPSDIAVEWESNGQPENNYKTTPPVLDSDGSFFLYSKLTVDKSRWQQGNVFSCSVMHEALHNHYTQKSLSLSPGK

SEQ ID NO: 69 - protein, 449 aa, synthetic construct
  source 1..449: note = heavy chain of anti-CSF3 antibody
QMQLVQSGAEARKPGSSVKVSCKASGYTFTNYGISWLRQTPGQGLEWMGWINPNSGGTIYAQKFQGRVTMTRDTSITTAYMELSTLRSEDTAVYYCSRGSGGTSPFDVWGQGTMVTVSSASTKGPSVFPLAPSSKSTSGGTAALGCLVKDYFPEPVTVSWNSGALTSGVHTFPAVLQSSGLYSLSSVVTVPSSSLGTQTYICNVNHKPSNTKVDKKVEPKSCDKTHTCPPCPAPELLGGPSVFLFPPKPKDTLMISRTPEVTCVVVDVSHEDPEVKFNWYVDGVEVHNAKTKPREEQYNSTYRVVSVLTVLHQDWLNGKEYKCKVSNKALPAPIEKTISKAKGQPREPQVYTLPPSREEMTKNQVSLTCLVKGFYPSDIAVEWESNGQPENNYKTTPPVLDSDGSFFLYSKLTVDKSRWQQGNVFSCSVMHEALHNHYTQKSLSLSPGK

SEQ ID NO: 70 - protein, 449 aa, synthetic construct
  source 1..449: note = heavy chain of anti-CSF3 antibody
QMQLVQSGAEARKPGSSVKVSCKASGYTFTNYGISWLRQTPGQGLEWMGWINPNSGGTIYAQKFQGRVTMTRDTSITTAYMELSTLRSEDTAVYYCSRGSGGIKPFDVWGQGTMVTVSSASTKGPSVFPLAPSSKSTSGGTAALGCLVKDYFPEPVTVSWNSGALTSGVHTFPAVLQSSGLYSLSSVVTVPSSSLGTQTYICNVNHKPSNTKVDKKVEPKSCDKTHTCPPCPAPELLGGPSVFLFPPKPKDTLMISRTPEVTCVVVDVSHEDPEVKFNWYVDGVEVHNAKTKPREEQYNSTYRVVSVLTVLHQDWLNGKEYKCKVSNKALPAPIEKTISKAKGQPREPQVYTLPPSREEMTKNQVSLTCLVKGFYPSDIAVEWESNGQPENNYKTTPPVLDSDGSFFLYSKLTVDKSRWQQGNVFSCSVMHEALHNHYTQKSLSLSPGK

SEQ ID NO: 71 - protein, 449 aa, synthetic construct
  source 1..449: note = heavy chain of anti-CSF3 antibody
EMQLVQSGAEARKPGSSVKVSCKASGYTFTNYGISWLRQTPGQGLEWMGWINPNSGGTIYAQKFQGRVTMTRDTPITTAYMELSTLRSEDTAVYYCSRGSGGAVPFDVWGQGTMVTVSSASTKGPSVFPLAPSSKSTSGGTAALGCLVKDYFPEPVTVSWNSGALTSGVHTFPAVLQSSGLYSLSSVVTVPSSSLGTQTYICNVNHKPSNTKVDKKVEPKSCDKTHTCPPCPAPELLGGPSVFLFPPKPKDTLMISRTPEVTCVVVDVSHEDPEVKFNWYVDGVEVHNAKTKPREEQYNSTYRVVSVLTVLHQDWLNGKEYKCKVSNKALPAPIEKTISKAKGQPREPQVYTLPPSREEMTKNQVSLTCLVKGFYPSDIAVEWESNGQPENNYKTTPPVLDSDGSFFLYSKLTVDKSRWQQGNVFSCSVMHEALHNHYTQKSLSLSPGK

SEQ ID NO: 72 - protein, 449 aa, synthetic construct
  source 1..449: note = heavy chain of anti-CSF3 antibody
QMQLVQSGAEARKPGSSVKVSCKASGYTFTNYGISWLRQTPGQGLEWMGWINPNSGGTIYAQKFQGRVTMTRDTSITTAYMELSTLRSEDTAVYYCSRGSGGIAPFDVWGQGTMVTVSSASTKGPSVFPLAPSSKSTSGGTAALGCLVKDYFPEPVTVSWNSGALTSGVHTFPAVLQSSGLYSLSSVVTVPSSSLGTQTYICNVNHKPSNTKVDKKVEPKSCDKTHTCPPCPAPELLGGPSVFLFPPKPKDTLMISRTPEVTCVVVDVSHEDPEVKFNWYVDGVEVHNAKTKPREEQYNSTYRVVSVLTVLHQDWLNGKEYKCKVSNKALPAPIEKTISKAKGQPREPQVYTLPPSREEMTKNQVSLTCLVKGFYPSDIAVEWESNGQPENNYKTTPPVLDSDGSFFLYSKLTVDKSRWQQGNVFSCSVMHEALHNHYTQKSLSLSPGK

SEQ ID NO: 73 - protein, 449 aa, synthetic construct
  source 1..449: note = heavy chain of anti-CSF3 antibody
QMQLVQSGAEARKPGSSVKVSCKASGYTFTNYGISWLRQTPGQGLEWMGWINPNSGGTIYAQKFQGRVTMTRDTSITTAYMELSTLRSEDTAVYYCSRGSGGLLPFDVWGQGTMVTVSSASTKGPSVFPLAPSSKSTSGGTAALGCLVKDYFPEPVTVSWNSGALTSGVHTFPAVLQSSGLYSLSSVVTVPSSSLGTQTYICNVNHKPSNTKVDKKVEPKSCDKTHTCPPCPAPELLGGPSVFLFPPKPKDTLMISRTPEVTCVVVDVSHEDPEVKFNWYVDGVEVHNAKTKPREEQYNSTYRVVSVLTVLHQDWLNGKEYKCKVSNKALPAPIEKTISKAKGQPREPQVYTLPPSREEMTKNQVSLTCLVKGFYPSDIAVEWESNGQPENNYKTTPPVLDSDGSFFLYSKLTVDKSRWQQGNVFSCSVMHEALHNHYTQKSLSLSPGK

SEQ ID NO: 74 - protein, 449 aa, synthetic construct
  source 1..449: note = heavy chain of anti-CSF3 antibody
QMQLVQSGAEARKPGSSVKVSCKASGYTFTNYGISWLRQTPGQGLEWMGWINPNSGGTIYAQKFQGRVTMTRDTSITTAYMELSTLRSEDTAVYYCSRGSGGMVPFDVWGQGTMVTVSSASTKGPSVFPLAPSSKSTSGGTAALGCLVKDYFPEPVTVSWNSGALTSGVHTFPAVLQSSGLYSLSSVVTVPSSSLGTQTYICNVNHKPSNTKVDKKVEPKSCDKTHTCPPCPAPELLGGPSVFLFPPKPKDTLMISRTPEVTCVVVDVSHEDPEVKFNWYVDGVEVHNAKTKPREEQYNSTYRVVSVLTVLHQDWLNGKEYKCKVSNKALPAPIEKTISKAKGQPREPQVYTLPPSREEMTKNQVSLTCLVKGFYPSDIAVEWESNGQPENNYKTTPPVLDSDGSFFLYSKLTVDKSRWQQGNVFSCSVMHEALHNHYTQKSLSLSPGK

SEQ ID NO: 75 - protein, 449 aa, synthetic construct
  source 1..449: note = heavy chain of anti-CSF3 antibody
QMQLVQSGAEARKPGSSVKVSCKASGYTFTNYGISWLRQTPGQGLEWMGWINPNSGGTIYAQKFQGRVTMTRDTSITTAYMELSTLRSEDTAVYYCSRGSGGRSGFDVWGQGTMVTVSSASTKGPSVFPLAPSSKSTSGGTAALGCLVKDYFPEPVTVSWNSGALTSGVHTFPAVLQSSGLYSLSSVVTVPSSSLGTQTYICNVNHKPSNTKVDKKVEPKSCDKTHTCPPCPAPELLGGPSVFLFPPKPKDTLMISRTPEVTCVVVDVSHEDPEVKFNWYVDGVEVHNAKTKPREEQYNSTYRVVSVLTVLHQDWLNGKEYKCKVSNKALPAPIEKTISKAKGQPREPQVYTLPPSREEMTKNQVSLTCLVKGFYPSDIAVEWESNGQPENNYKTTPPVLDSDGSFFLYSKLTVDKSRWQQGNVFSCSVMHEALHNHYTQKSLSLSPGK

SEQ ID NO: 76 - protein, 449 aa, synthetic construct
  source 1..449: note = heavy chain of anti-CSF3 antibody
QMQLVQSGAEARKPGSSVKVSCKASGYTFTNYGISWLRQTPGQGLEWMGWINPNSGGTIYAQKFQGRVTMTRDTSITTAYMELSTLRSEDTAVYYCSRGSGGFQAFDVWGQGTMVTVSSASTKGPSVFPLAPSSKSTSGGTAALGCLVKDYFPEPVTVSWNSGALTSGVHTFPAVLQSSGLYSLSSVVTVPSSSLGTQTYICNVNHKPSNTKVDKKVEPKSCDKTHTCPPCPAPELLGGPSVFLFPPKPKDTLMISRTPEVTCVVVDVSHEDPEVKFNWYVDGVEVHNAKTKPREEQYNSTYRVVSVLTVLHQDWLNGKEYKCKVSNKALPAPIEKTISKAKGQPREPQVYTLPPSREEMTKNQVSLTCLVKGFYPSDIAVEWESNGQPENNYKTTPPVLDSDGSFFLYSKLTVDKSRWQQGNVFSCSVMHEALHNHYTQKSLSLSPGK

SEQ ID NO: 77 - protein, 449 aa, synthetic construct
  source 1..449: note = heavy chain of anti-CSF3 antibody
QMQLVQSGAEARKPGSSVKVSCKASGYTFTNYGISWLRQTPGQGLEWMGWINPNSGGTIYAQKFQGRVTMTRDTSITTAYMELSTLRSEDTAVYYCSRGSGGLVPFDVWGQGTMVTVSSASTKGPSVFPLAPSSKSTSGGTAALGCLVKDYFPEPVTVSWNSGALTSGVHTFPAVLQSSGLYSLSSVVTVPSSSLGTQTYICNVNHKPSNTKVDKKVEPKSCDKTHTCPPCPAPELLGGPSVFLFPPKPKDTLMISRTPEVTCVVVDVSHEDPEVKFNWYVDGVEVHNAKTKPREEQYNSTYRVVSVLTVLHQDWLNGKEYKCKVSNKALPAPIEKTISKAKGQPREPQVYTLPPSREEMTKNQVSLTCLVKGFYPSDIAVEWESNGQPENNYKTTPPVLDSDGSFFLYSKLTVDKSRWQQGNVFSCSVMHEALHNHYTQKSLSLSPGK

SEQ ID NO: 78 - protein, 449 aa, synthetic construct
  source 1..449: note = heavy chain of anti-CSF3 antibody
QMQLVQSGAEARKPGSSVKVSCKASGYTFTNYGISWLRQTPGQGLEWMGWINPNSGGTIYAQKFQGRVTMTRDTSITTAYMELSTLRSEDTAVYYCSRGSGGIRPFDVWGQGTMVTVSSASTKGPSVFPLAPSSKSTSGGTAALGCLVKDYFPEPVTVSWNSGALTSGVHTFPAVLQSSGLYSLSSVVTVPSSSLGTQTYICNVNHKPSNTKVDKKVEPKSCDKTHTCPPCPAPELLGGPSVFLFPPKPKDTLMISRTPEVTCVVVDVSHEDPEVKFNWYVDGVEVHNAKTKPREEQYNSTYRVVSVLTVLHQDWLNGKEYKCKVSNKALPAPIEKTISKAKGQPREPQVYTLPPSREEMTKNQVSLTCLVKGFYPSDIAVEWESNGQPENNYKTTPPVLDSDGSFFLYSKLTVDKSRWQQGNVFSCSVMHEALHNHYTQKSLSLSPGK

SEQ ID NO: 79 - protein, 449 aa, synthetic construct
  source 1..449: note = heavy chain of anti-CSF3 antibody
QMQLVQSGAEARKPGSSVKVSCKASGYTFTNYGISWLRQTPGQGLEWMGWINPNSGGTIYAQKFQGRVTMTRDTSITTAYMELSTLRSEDTAVYYCSRGSGGFFPFDVWGQGTMVTVSSASTKGPSVFPLAPSSKSTSGGTAALGCLVKDYFPEPVTVSWNSGALTSGVHTFPAVLQSSGLYSLSSVVTVPSSSLGTQTYICNVNHKPSNTKVDKKVEPKSCDKTHTCPPCPAPELLGGPSVFLFPPKPKDTLMISRTPEVTCVVVDVSHEDPEVKFNWYVDGVEVHNAKTKPREEQYNSTYRVVSVLTVLHQDWLNGKEYKCKVSNKALPAPIEKTISKAKGQPREPQVYTLPPSREEMTKNQVSLTCLVKGFYPSDIAVEWESNGQPENNYKTTPPVLDSDGSFFLYSKLTVDKSRWQQGNVFSCSVMHEALHNHYTQKSLSLSPGK

SEQ ID NO: 80 - protein, 449 aa, synthetic construct
  source 1..449: note = heavy chain of anti-CSF3 antibody
QMQLVQSGAEARKPGSSVKVSCKASGYTFTNYGISWLRQTPGQGLEWMGWINPNSGGTIYAQKFQGRVTMTRDTSITTAYMELSTLRSEDTAVYYCSRGSGGYSGFDVWGQGTMVTVSSASTKGPSVFPLAPSSKSTSGGTAALGCLVKDYFPEPVTVSWNSGALTSGVHTFPAVLQSSGLYSLSSVVTVPSSSLGTQTYICNVNHKPSNTKVDKKVEPKSCDKTHTCPPCPAPELLGGPSVFLFPPKPKDTLMISRTPEVTCVVVDVSHEDPEVKFNWYVDGVEVHNAKTKPREEQYNSTYRVVSVLTVLHQDWLNGKEYKCKVSNKALPAPIEKTISKAKGQPREPQVYTLPPSREEMTKNQVSLTCLVKGFYPSDIAVEWESNGQPENNYKTTPPVLDSDGSFFLYSKLTVDKSRWQQGNVFSCSVMHEALHNHYTQKSLSLSPGK

SEQ ID NO: 81 - protein, 214 aa, synthetic construct
  source 1..214: note = light chain of anti-CSF3 antibody
DIQMTQSPFSLSASVGDRVTITCRASQTISTYLNWYQHKPGKAPKLFIYYASSLQSGVPSRFSGSGSGTDFALTISSLQPEDFATYYCQQGYSSPRTFGQGTKVEIKRTVAAPSVFIFPPSDEQLKSGTASVVCLLNNFYPREAKVQWKVDNALQSGNSQESVTEQDSKDSTYSLSSTLTLSKADYEKHKVYACEVTHQGLSSPVTKSFNRGEC

SEQ ID NO: 82 - protein, 214 aa, synthetic construct
  source 1..214: note = light chain of anti-CSF3 antibody
DIQMTQSPFSLSASVGDRVTITCRASQTISTYLNWYQHKPGKAPKLFIYYASSLQSGVPSRFSGSGSGTDFALTISSLQPEDFATYYCQQGYSSPRTFGQGTKVEITRTVAAPSVFIFPPSDEQLKSGTASVVCLLNNFYPREAKVQWKVDNALQSGNSQESVTEQDSKDSTYSLSSTLTLSKADYEKHKVYACEVTHQGLSSPVTKSFNRGEC

SEQ ID NO: 83 - protein, 214 aa, synthetic construct
  source 1..214: note = light chain of anti-CSF3 antibody
DIQMTQSPFSLSASVGDRVTITCRASQTTGQYLNWYQHKPGKAPKLFIYYASSLQSGVPSRFSGSGSGTDFALTISSLQPEDFATYYCQQGYSSPRTFGQGTKVEIKRTVAAPSVFIFPPSDEQLKSGTASVVCLLNNFYPREAKVQWKVDNALQSGNSQESVTEQDSKDSTYSLSSTLTLSKADYEKHKVYACEVTHQGLSSPVTKSFNRGEC

SEQ ID NO: 84 - protein, 214 aa, synthetic construct
  source 1..214: note = light chain of anti-CSF3 antibody
DIQMTQSPFSLSASVGDRVTITCRASQTISNRLNWYQHKPGKAPKLFIYYASSLQSGVPSRFSGSGSGTDFALTISSLQPEDFATYYCQQGYSSPRTFGQGTKVEIKRTVAAPSVFIFPPSDEQLKSGTASVVCLLNNFYPREAKVQWKVDNALQSGNSQESVTEQDSKDSTYSLSSTLTLSKADYEKHKVYACEVTHQGLSSPVTKSFNRGEC

SEQ ID NO: 85 - protein, 214 aa, synthetic construct
  source 1..214: note = light chain of anti-CSF3 antibody
DIQMTQSPFSLSASVGDRVTITCRASKSISTYLNWYQHKPGKAPKLFIYYASSLQSGVPSRFSGSGSGTDFALTISSLQPEDFATYYCQQGYSSPRTFGQGTKVEIKRTVAAPSVFIFPPSDEQLKSGTASVVCLLNNFYPREAKVQWKVDNALQSGNSQESVTEQDSKDSTYSLSSTLTLSKADYEKHKVYACEVTHQGLSSPVTKSFNRGEC

SEQ ID NO: 86 - protein, 204 aa, Homo sapiens
  source 1..204: note = human CSF3 protein
MAGPATQSPMKLMALQLLLWHSALWTVQEATPLGPASSLPQSFLLKCLEQVRKIQGDGAALQEKLCATYKLCHPEELVLLGHSLGIPWAPLSSCPSQALQLAGCLSQLHSGLFLYQGLLQALEGISPELGPTLDTLQLDVADFATTIWQQMEELGMAPALQPTQGAMPAFASAFQRRAGGVLVASHLQSFLEVSYRVLRHLAQP

SEQ ID NO: 87 - protein, 10 aa, synthetic construct
  source 1..10: note = epitope of CSF3 protein
KLCATYKLCH

SEQ ID NO: 88 - protein, 4 aa, synthetic construct
  source 1..4: note = epitope of CSF3 protein
TLDT

SEQ ID NO: 89 - protein, 5 aa, synthetic construct
  source 1..5: note = epitope of CSF3 protein
SAFQR

SEQ ID NO: 90 - protein, 6 aa, synthetic construct
  source 1..6: note = epitope of CSF3 protein
SAFQRR

SEQ ID NO: 91 - protein, 8 aa, synthetic construct
  source 1..8: note = CDRH1 of surrogate antibody
GYTFTSYD

SEQ ID NO: 92 - protein, 8 aa, synthetic construct
  source 1..8: note = CDRH2 of surrogate antibody
IYPGDGST

SEQ ID NO: 93 - protein, 8 aa, synthetic construct
  source 1..8: note = CDRH3 of surrogate antibody
ARGGWFAY

SEQ ID NO: 94 - protein, 12 aa, synthetic construct
  source 1..12: note = CDRL1 of surrogate antibody
QSLLNSRTRKNY

SEQ ID NO: 95 - skipped

SEQ ID NO: 96 - protein, 8 aa, synthetic construct
  source 1..8: note = CDRL3 of surrogate antibody
KQSYNLYT

SEQ ID NO: 97 - protein, 115 aa, synthetic construct
  source 1..115: note = heavy chain of surrogate antibody
QVQLKQSGPELVKPGALVKISCKASGYTFTSYDINWVKQRPGQGLEWIGWIYPGDGSTKYNEKFKGKATLTADKSSSTAYMQLSSLTSENSAVYFCARGGWFAYWGQGTLVTVSA

SEQ ID NO: 98 - protein, 112 aa, synthetic construct
  source 1..112: note = light chain of surrogate antibody
DIVMTQSPSSLAVSAGEKVTMSCKSSQSLLNSRTRKNYLAWYQQKPGQSPKLLIYWASTRESGVPDRFTGSGSGTDFTLTISSVQAEDLAVYYCKQSYNLYTFGGGTKLEIK

SEQ ID NO: 99 - RNA, 615 nt, Homo sapiens
  source 1..615: mol_type = genomic RNA; note = mRNA of human CSF3
atggctggacctgccacccagagccccatgaagctgatggccctgcagctgctgctgtggcacagtgcactctggacagtgcaggaagccacccccctgggccctgccagctccctgccccagagcttcctgctcaagtgcttagagcaagtgaggaagatccagggcgatggcgcagcgctccaggagaagctgtgtgccacctacaagctgtgccaccccgaggagctggtgctgctcggacactctctgggcatcccctgggctcccctgagcagctgccccagccaggccctgcagctggcaggctgcttgagccaactccatagcggccttttcctctaccaggggctcctgcaggccctggaagggatctcccccgagttgggtcccaccttggacacactgcagctggacgtcgccgactttgccaccaccatctggcagcagatggaagaactgggaatggcccctgccctgcagcccacccagggtgccatgccggccttcgcctctgctttccagcgccgggcaggaggggtcctggttgcctcccatctgcagagcttcctggaggtgtcgtaccgcgttctacgccaccttgcccagccctga

SEQ ID NO: 100 - DNA, 21 bp, synthetic construct
  source 1..21: mol_type = other DNA; note = primer against a-SMA
aatcccatcaccatcttccag

SEQ ID NO: 101 - DNA, 21 bp, synthetic construct
  source 1..21: mol_type = other DNA; note = primer against a-SMA
gcagtggccatctcattttca

SEQ ID NO: 102 - DNA, 20 bp, synthetic construct
  source 1..20: mol_type = other DNA; note = primer against collagen
cctggatgccatcaaagtct

SEQ ID NO: 103 - DNA, 20 bp, synthetic construct
  source 1..20: mol_type = other DNA; note = primer against collagen
aatccatcggtcatgctctc

SEQ ID NO: 104 - DNA, 20 bp, synthetic construct
  source 1..20: mol_type = other DNA; note = primer against CSF3
gctgcttgagccaactccat

SEQ ID NO: 105 - DNA, 23 bp, synthetic construct
  source 1..23: mol_type = other DNA; note = primer against CSF3
cattcccagttcttccatctgct

SEQ ID NO: 106 - DNA, 19 bp, synthetic construct
  source 1..19: mol_type = other DNA; note = primer against CSF3R
cagatacgctgcatccgct

SEQ ID NO: 107 - DNA, 20 bp, synthetic construct
  source 1..20: mol_type = other DNA; note = primer against CSF3R
cactggcttccagaacagct

SEQ ID NO: 108 - DNA, 19 bp, synthetic construct
  source 1..19: mol_type = other DNA; note = primer against TGF-b
cccagcatctgcaaagctc

SEQ ID NO: 109 - DNA, 20 bp, synthetic construct
  source 1..20: mol_type = other DNA; note = primer against TGF-b
gtcaatgtacagctgccgca

SEQ ID NO: 110 - DNA, 20 bp, synthetic construct
  source 1..20: mol_type = other DNA; note = primer against IL-11
acagctgagggacaaattcc

SEQ ID NO: 111 - DNA, 19 bp, synthetic construct
  source 1..19: mol_type = other DNA; note = primer against IL-11
agcacacctgggagctgta

SEQ ID NO: 112 - DNA, 21 bp, synthetic construct
  source 1..21: mol_type = other DNA; note = primer against GAPDH
aatcccatcaccatcttccag

SEQ ID NO: 113 - DNA, 18 bp, synthetic construct
  source 1..18: mol_type = other DNA; note = primer against GAPDH
aaatgagccccagccttc

SEQ ID NO: 114 - RNA, 19 nt, synthetic construct
  source 1..19: mol_type = other RNA; note = siRNA1 against CSF3
gtttgactcccgaacatca

SEQ ID NO: 115 - RNA, 19 nt, synthetic construct
  source 1..19: mol_type = other RNA; note = siRNA1 against CSF3
tgatgttcgggagtcaaac

SEQ ID NO: 116 - RNA, 19 nt, synthetic construct
  source 1..19: mol_type = other RNA; note = siRNA2 against CSF3
ccatctggcagcagatgga

SEQ ID NO: 117 - RNA, 19 nt, synthetic construct
  source 1..19: mol_type = other RNA; note = siRNA2 against CSF3
tccatctgctgccagatgg

SEQ ID NO: 118 - RNA, 19 nt, synthetic construct
  source 1..19: mol_type = other RNA; note = siRNA3 against CSF3
ggtgtcgtaccgcgttcta

SEQ ID NO: 119 - RNA, 19 nt, synthetic construct
  source 1..19: mol_type = other RNA; note = siRNA3 against CSF3
tagaacgcggtacgacacc

SEQ ID NO: 120 - DNA, 48 bp, synthetic construct
  source 1..48: mol_type = other DNA; note = CSF3-C-6xHis-Forward
tggtggccacagcggccgatgtccactcgacccccctgggccctgcca

SEQ ID NO: 121 - DNA, 51 bp, synthetic construct
  source 1..51: mol_type = other DNA; note = CSF3-C-6xHis--Reverse
aattctcgagtcagtggtgatgatggtgatggggctgggcaaggtggcgta

SEQ ID NO: 122 - DNA, 48 bp, synthetic construct; identical to SEQ ID NO: 120
  source 1..48: mol_type = other DNA; note = CSF3-C-Fc-Forward

SEQ ID NO: 123 - DNA, 28 bp, synthetic construct
  source 1..28: mol_type = other DNA; note = CSF3-C-Fc- Reverse
aagctagcgggctgggcaaggtggcgta

SEQ ID NO: 124 - protein, 8 aa, synthetic construct
  source 1..8: note = CDRH1 of anti-CSF3R antibody
GFIFSNYA

SEQ ID NO: 125 - protein, 8 aa, synthetic construct
  source 1..8: note = CDRH2 of anti-CSF3R antibody
INGNGGVT

SEQ ID NO: 126 - protein, 11 aa, synthetic construct
  source 1..11: note = CDRH3 of anti-CSF3R antibody
ARESAMYGMDV

SEQ ID NO: 127 - protein, 6 aa, synthetic construct
  source 1..6: note = CDRL1 of anti-CSF3R antibody
QSILTY

SEQ ID NO: 128 - skipped

SEQ ID NO: 129 - protein, 9 aa, synthetic construct
  source 1..9: note = CDRL3 of anti-CSF3R antibody
QQSYSSPYS

SEQ ID NO: 130 - protein, 118 aa, synthetic construct
  source 1..118: note = VH of anti-CSF3R antibody
QMQLVQSGGGLVQPGGSLRLSCAASGFIFSNYAMNWVRQAPGKGLEWVSTINGNGGVTYYADSVKGRFTISRDNSKNSLYLQMNSLRAEDTAVYYCARESAMYGMDVWGQGTTVTVSS

SEQ ID NO: 131 - protein, 107 aa, synthetic construct
  source 1..107: note = VL of anti-CSF3R antibody
DIVMTQTPLSLSASVGDRLTITCRASQSILTYLNWYQQKPGKAPKLLVYAASSLQRGVPSRFSGRGSGTDFTLTISGLQPDDFALYYCQQSYSSPYSFGPGTKVDIK

SEQ ID NO: 132 - protein, 448 aa, synthetic construct
  source 1..448: note = heavy chain of anti-CSF3R antibody
QMQLVQSGGGLVQPGGSLRLSCAASGFIFSNYAMNWVRQAPGKGLEWVSTINGNGGVTYYADSVKGRFTISRDNSKNSLYLQMNSLRAEDTAVYYCARESAMYGMDVWGQGTTVTVSSASTKGPSVFPLAPSSKSTSGGTAALGCLVKDYFPEPVTVSWNSGALTSGVHTFPAVLQSSGLYSLSSVVTVPSSSLGTQTYICNVNHKPSNTKVDKKVEPKSCDKTHTCPPCPAPELLGGPSVFLFPPKPKDTLMISRTPEVTCVVVDVSHEDPEVKFNWYVDGVEVHNAKTKPREEQYNSTYRVVSVLTVLHQDWLNGKEYKCKVSNKALPAPIEKTISKAKGQPREPQVYTLPPSREEMTKNQVSLTCLVKGFYPSDIAVEWESNGQPENNYKTTPPVLDSDGSFFLYSKLTVDKSRWQQGNVFSCSVMHEALHNHYTQKSLSLSPGK

SEQ ID NO: 133 - protein, 214 aa, synthetic construct
  source 1..214: note = light chain of anti-CSF3R antibody
DIVMTQTPLSLSASVGDRLTITCRASQSILTYLNWYQQKPGKAPKLLVYAASSLQRGVPSRFSGRGSGTDFTLTISGLQPDDFALYYCQQSYSSPYSFGPGTKVDIKRTVAAPSVFIFPPSDEQLKSGTASVVCLLNNFYPREAKVQWKVDNALQSGNSQESVTEQDSKDSTYSLSSTLTLSKADYEKHKVYACEVTHQGLSSPVTKSFNRGEC

SEQ ID NO: 134 - protein, 5 aa, synthetic construct
  source 1..5: note = peptide fragment derived from anti-CSF3 antibody
YASSL

SEQ ID NO: 135 - protein, 20 aa, synthetic construct
  source 1..20: note = peptide fragment derived from human CSF3 protein
KCLEQVRKIQGDGAALQEKL

SEQ ID NO: 136 - protein, 13 aa, synthetic construct
  source 1..13: note = peptide fragment derived from anti-CSF3 antibody
MGWINPNSGGTIY

SEQ ID NO: 137 - protein, 10 aa, synthetic construct
  source 1..10: note = peptide fragment derived from human CSF3 protein
ATYKLCHPEE

SEQ ID NO: 138 - protein, 10 aa, synthetic construct
  source 1..10: note = peptide fragment derived from anti-CSF3 antibody
KAPKLFIYYA

SEQ ID NO: 139 - protein, 7 aa, synthetic construct
  source 1..7: note = peptide fragment derived from human CSF3 protein
CHPEELV

SEQ ID NO: 140 - protein, 13 aa, synthetic construct
  source 1..13: note = peptide fragment derived from anti-CSF3 antibody
MGWINPNSGGTIY

SEQ ID NO: 141 - protein, 8 aa, synthetic construct
  source 1..8: note = peptide fragment derived from human CSF3 protein
LCHPEELV

SEQ ID NO: 142 - protein, 15 aa, synthetic construct
  source 1..15: note = peptide fragment derived from anti-CSF3 antibody
EWMGWINPNSGGTIY

SEQ ID NO: 143 - protein, 8 aa, synthetic construct
  source 1..8: note = peptide fragment derived from human CSF3 protein
KLCHPEEL

SEQ ID NO: 144 - protein, 27 aa, synthetic construct
  source 1..27: note = peptide fragment derived from anti-CSF3 antibody
EWMGWINPNSGGTIYAQKFQGRVTMTR

SEQ ID NO: 145 - protein, 6 aa, synthetic construct
  source 1..6: note = peptide fragment derived from human CSF3 protein
ELGPTL

SEQ ID NO: 146 - protein, 20 aa, synthetic construct
  source 1..20: note = peptide fragment derived from anti-CSF3 antibody
ATYYCQQGYSSPRTFGQGTK

SEQ ID NO: 147 - protein, 7 aa, synthetic construct
  source 1..7: note = peptide fragment derived from human CSF3 protein
LDTLQLD

SEQ ID NO: 148 - protein, 22 aa, synthetic construct
  source 1..22: note = peptide fragment derived from anti-CSF3 antibody
ATYYCQQGYSSPRTFGQGTKVE

SEQ ID NO: 149 - protein, 5 aa, synthetic construct
  source 1..5: note = peptide fragment derived from human CSF3 protein
LDTLQ

SEQ ID NO: 150 - protein, 17 aa, synthetic construct
  source 1..17: note = peptide fragment derived from anti-CSF3 antibody
MGWINPNSGGTIYAQKF

SEQ ID NO: 151 - protein, 22 aa, synthetic construct
  source 1..22: note = peptide fragment derived from human CSF3 protein
QPTQGAMPAFASAFQRRAGGVL

SEQ ID NO: 152 - protein, 20 aa, synthetic construct
  source 1..20: note = peptide fragment derived from anti-CSF3 antibody
ATYYCQQGYSSPRTFGQGTK

SEQ ID NO: 153 - protein, 8 aa, synthetic construct
  source 1..8: note = peptide fragment derived from human CSF3 protein
AFQRRAGG

SEQ ID NO: 154 - protein, 22 aa, synthetic construct
  source 1..22: note = peptide fragment derived from anti-CSF3 antibody
ATYYCQQGYSSPRTFGQGTKVE

SEQ ID NO: 155 - protein, 8 aa, synthetic construct
  source 1..8: note = peptide fragment derived from human CSF3 protein
AFQRRAGG

SEQ ID NO: 156 - protein, 8 aa, synthetic construct
  source 1..8: note = peptide fragment derived from anti-CSF3 antibody
ASQTISNR

SEQ ID NO: 157 - protein, 8 aa, synthetic construct
  source 1..8: note = peptide fragment derived from human CSF3 protein
AFQRRAGG

SEQ ID NO: 158 - protein, 15 aa, synthetic construct
  source 1..15: note = peptide fragment derived from anti-CSF3 antibody
ASGYTFTNYGISWLR

SEQ ID NO: 159 - protein, 20 aa, synthetic construct
  source 1..20: note = peptide fragment derived from human CSF3 protein
RAGGVLVASHLQSFLEVSYR

SEQ ID NO: 160 - protein, 20 aa, synthetic construct
  source 1..20: note = peptide fragment derived from anti-CSF3 antibody
CQQGYSSPRTFGQGTKVEIK

SEQ ID NO: 161 - protein, 13 aa, synthetic construct
  source 1..13: note = peptide fragment derived from human CSF3 protein
QRRAGGVLVASHL

SEQ ID NO: 162 - protein, 15 aa, synthetic construct
  source 1..15: note = peptide fragment derived from anti-CSF3 antibody
ASGYTFTNYGISWLR

SEQ ID NO: 163 - protein, 20 aa, synthetic construct
  source 1..20: note = peptide fragment derived from human CSF3 protein
RAGGVLVASHLQSFLEVSYR